European Patent Application EP 4 524 251 A1, published March 19, 2025. Title: INHIBITORY NEURON-SPECIFIC PROMOTER. Applicant: NATIONAL UNIVERSITY CORPORATION GUNMA UNIVERSITY. Application EP. The sequence listing filed with the application follows.

SEQUENCE LISTING (50 sequences)

SEQ ID NO: 1 - DNA, 206 bp, Mus musculus
  source 1..206: mol_type = genomic DNA
tttctgggtggctcacagtggacaaggaataggtaatcccaccaaaccttgaggtgggctaaactggagattttggtatgggtctcctactgtaaagagaaagccttccgggctaacggtattcctttcgcagtctactgcctcctttgtgaactaatgactgtaattattacctcccagagctcttttgttatcaacaacccgga

SEQ ID NO: 2 - DNA, 361 bp, Mus musculus
  source 1..361: mol_type = genomic DNA
aaaagggaaacagaaaggattttttcattcctttattagaaaacacaaacgaaactacttctttctgggctgggaaattgccactgttgtgttcctaggcacctgctgatggcaagaactcctcttgggaagggacgaggtcagtgggttgagtatccctgaaaagatgggagtgccttttcctgggatttggaaaaactgattcgcttactttgagactccctgaatcctgtgtatgtgtcagctctcacccactccaagaagtttctgttcgttttatttatttaatttttctcagcctgaggtcctcagtgatagattccagcgtggattttaattgcttcaatcagcagcctttctc

SEQ ID NO: 3 - DNA, 122 bp, Mus musculus
  source 1..122: mol_type = genomic DNA
cgcctgtggctgggtcagcactacgcaggcacgcctccctcccccgcatctgactcgcacctcacgacccagcgcctccatttcccttccgtcactctctcatctccccaccaagctccctc

SEQ ID NO: 4 - DNA, 1177 bp, synthetic construct
  misc_feature 1..1177: note = mGAD65(Ri-Rii-D-ETSS)
  source 1..1177: mol_type = other DNA
tcgagatttctgggtggctcacagtggacaaggaataggtaatcccaccaaaccttgaggtgggctaaactggagattttggtatgggtctcctactgtaaagagaaagccttccgggctaacggtattcctttcgcagtctactgcctcctttgtgaactaatgactgtaattattacctcccagagctcttttgttatcaacaacccggaggaaaagggaaacagaaaggattttttcattcctttattagaaaacacaaacgaaactacttctttctgggctgggaaattgccactgttgtgttcctaggcacctgctgatggcaagaactcctcttgggaagggacgaggtcagtgggttgagtatccctgaaaagatgggagtgccttttcctgggatttggaaaaactgattcgcttactttgagactccctgaatcctgtgtatgtgtcagctctcacccactccaagaagtttctgttcgttttatttatttaatttttctcagcctgaggtcctcagtgatagattccagcgtggattttaattgcttcaatcagcagcctttctcttcagccgtcagtcaaaacctggacgatgggtctggggacccaggcatgactgcacagaaaccgtacgacccccacccccaccccccaggctggctcagctcagcaggcagacattaggctctgctaaggagatgaaatgagttcgttggtgtggaagcggtccaccttcctccctccttggttccttccccaagctttggagctcttcctgattgaggccaggtggcctgggctcttgaggtcacagcgacctcagcactggtttggaggaaggcgggcgcgagaaccacttttgctcggcagcagccagagacagccctcaaacaatgagccaatcgatgcacacgtgaaattgccctcggccaccattccaatcttgccaaggtctccctgtccctggggtcacctaggccagcgtgctgagggctgtggtagcaccctggacagcgcgttccggcagaagcagacctggagcgcctgtggctgggtcagcactacgcaggcacgcctccctcccccgcatctgactcgcacctcacgacccagcgcctccatttcccttccgtcactctctcatctccccaccaagctccctcaccgg

SEQ ID NO: 5 - DNA, 704 bp, synthetic construct
  misc_feature 1..704: note = mGAD65(Ri-Rii-ETSS)
  source 1..704: mol_type = other DNA
tcgagatttctgggtggctcacagtggacaaggaataggtaatcccaccaaaccttgaggtgggctaaactggagattttggtatgggtctcctactgtaaagagaaagccttccgggctaacggtattcctttcgcagtctactgcctcctttgtgaactaatgactgtaattattacctcccagagctcttttgttatcaacaacccggaggaaaagggaaacagaaaggattttttcattcctttattagaaaacacaaacgaaactacttctttctgggctgggaaattgccactgttgtgttcctaggcacctgctgatggcaagaactcctcttgggaagggacgaggtcagtgggttgagtatccctgaaaagatgggagtgccttttcctgggatttggaaaaactgattcgcttactttgagactccctgaatcctgtgtatgtgtcagctctcacccactccaagaagtttctgttcgttttatttatttaatttttctcagcctgaggtcctcagtgatagattccagcgtggattttaattgcttcaatcagcagcctttctcttcgcctgtggctgggtcagcactacgcaggcacgcctccctcccccgcatctgactcgcacctcacgacccagcgcctccatttcccttccgtcactctctcatctccccaccaagctccctcaccgg

SEQ ID NO: 6 - DNA, 496 bp, synthetic construct
  misc_feature 1..496: note = mGAD65(Rii-ETSS)
  source 1..496: mol_type = other DNA
tcgaggaaaagggaaacagaaaggattttttcattcctttattagaaaacacaaacgaaactacttctttctgggctgggaaattgccactgttgtgttcctaggcacctgctgatggcaagaactcctcttgggaagggacgaggtcagtgggttgagtatccctgaaaagatgggagtgccttttcctgggatttggaaaaactgattcgcttactttgagactccctgaatcctgtgtatgtgtcagctctcacccactccaagaagtttctgttcgttttatttatttaatttttctcagcctgaggtcctcagtgatagattccagcgtggattttaattgcttcaatcagcagcctttctcttcgcctgtggctgggtcagcactacgcaggcacgcctccctcccccgcatctgactcgcacctcacgacccagcgcctccatttcccttccgtcactctctcatctccccaccaagctccctcaccgg

SEQ ID NO: 7 - DNA, 275 bp, Mus musculus
  source 1..275: mol_type = genomic DNA
ttcaccccgctcagtaatgtgcttaaatattgccaagagagaatcattgaacagcgtgaaactgaaaagaagcgaggagagcgggccaagacacggagtgccgtcctggcttcccggagccaccctccatgctctgctgccccaggcgtgtggagcggcactcgtgcgtgttattaaccttcagacatgatcaattacgaagatttcttttacccctctccagggagagggctcagagaaagggaaatagaccccttgcctcttgtggtgccagg

SEQ ID NO: 8 - DNA, 269 bp, Mus musculus
  source 1..269: mol_type = genomic DNA
acaaaattcttcgtaggaattatattttcccttgccctcacccaacatcgcctatctcaaaaataatttaaaaacaaaaaacaaacaaacaaacaaaaaacagagcgtgctgagtgcattctggattactcataggactttgtcacacacaccctcctttctggtcgcaaacccgtgagctggatttataatcgccctacaaagctccagaggcagtcagacacctgcaaaggagccccagcgctccgcggacgagctgcccccgcgag

SEQ ID NO: 9 - DNA, 172 bp, Mus musculus
  source 1..172: mol_type = genomic DNA
cagcgctccgcggacgagctgcccccgcgagcaacggcctcgtgattccccccgccgagcgggtccccgcctccccactccgcccccgcctcccccaagcccagcggccgcctctccggatctctcccttcttcaggctctcccgtgccggaccagggatcgtgcaagcaag

SEQ ID NO: 10 - DNA, 977 bp, synthetic construct
  misc_feature 1..977: note = mGAD67(Ri-M-Rii-ETSS)
  source 1..977: mol_type = other DNA
tcgagcttcaccccgctcagtaatgtgcttaaatattgccaagagagaatcattgaacagcgtgaaactgaaaagaagcgaggagagcgggccaagacacggagtgccgtcctggcttcccggagccaccctccatgctctgctgccccaggcgtgtggagcggcactcgtgcgtgttattaaccttcagacatgatcaattacgaagatttcttttacccctctccagggagagggctcagagaaagggaaatagaccccttgcctcttgtggtgccaggtagctgtgttcgaacgaggtagtgtggagatggactggaagaagaaacgggagtgcagaaactccagggtctgtctgggtggtcccctcatctccgctttgcctgtacagccatactggctcagtagagcgctccctaggacaccacccagagaaaaccttctggaatcgccaatccaggacaaccacaggagattgatcaaggcaaagcaaatattctagtcttctccaagatacgggatggagggctaggaagaggggaaggaagaatcacccagtgagacaaaattcttcgtaggaattatattttcccttgccctcacccaacatcgcctatctcaaaaataatttaaaaacaaaaaacaaacaaacaaacaaaaaacagagcgtgctgagtgcattctggattactcataggactttgtcacacacaccctcctttctggtcgcaaacccgtgagctggatttataatcgccctacaaagctccagaggcagtcagacacctgcaaaggagccccagcgctccgcggacgagctgcccccgcgagcaacggcctcgtgattccccccgccgagcgggtccccgcctccccactccgcccccgcctcccccaagcccagcggccgcctctccggatctctcccttcttcaggctctcccgtgccggaccagggatcgtgcaagcaagaccgg

SEQ ID NO: 11 - DNA, 698 bp, synthetic construct
  misc_feature 1..698: note = mGAD67(Ri-Rii-ETSS)
  source 1..698: mol_type = other DNA
tcgagcttcaccccgctcagtaatgtgcttaaatattgccaagagagaatcattgaacagcgtgaaactgaaaagaagcgaggagagcgggccaagacacggagtgccgtcctggcttcccggagccaccctccatgctctgctgccccaggcgtgtggagcggcactcgtgcgtgttattaaccttcagacatgatcaattacgaagatttcttttacccctctccagggagagggctcagagaaagggaaatagaccccttgcctcttgtggtgccaggtgacaaaattcttcgtaggaattatattttcccttgccctcacccaacatcgcctatctcaaaaataatttaaaaacaaaaaacaaacaaacaaacaaaaaacagagcgtgctgagtgcattctggattactcataggactttgtcacacacaccctcctttctggtcgcaaacccgtgagctggatttataatcgccctacaaagctccagaggcagtcagacacctgcaaaggagccccagcgctccgcggacgagctgcccccgcgagcaacggcctcgtgattccccccgccgagcgggtccccgcctccccactccgcccccgcctcccccaagcccagcggccgcctctccggatctctcccttcttcaggctctcccgtgccggaccagggatcgtgcaagcaagaccgg

SEQ ID NO: 12 - DNA, 420 bp, synthetic construct
  misc_feature 1..420: note = mGAD67(Rii-ETSS)
  source 1..420: mol_type = other DNA
tcgagacaaaattcttcgtaggaattatattttcccttgccctcacccaacatcgcctatctcaaaaataatttaaaaacaaaaaacaaacaaacaaacaaaaaacagagcgtgctgagtgcattctggattactcataggactttgtcacacacaccctcctttctggtcgcaaacccgtgagctggatttataatcgccctacaaagctccagaggcagtcagacacctgcaaaggagccccagcgctccgcggacgagctgcccccgcgagcaacggcctcgtgattccccccgccgagcgggtccccgcctccccactccgcccccgcctcccccaagcccagcggccgcctctccggatctctcccttcttcaggctctcccgtgccggaccagggatcgtgcaagcaagaccgg

SEQ ID NO: 13 - DNA, 2542 bp, Mus musculus
  source 1..2542: mol_type = genomic DNA
gctttgcttcctgggcactacagccccacctgaagcaggtgcgttagggaggagttgggctctgcagcttgccagattttaattctggcttccagcggaggaccctgcaccccacggtcctcgcaagagtgtctgggaaggtttattcggttgctgagtagagacgcaacagacagatctacctcagcccctgcaccttggcttgataaggctggaaaaggaagattgcaacgtcgtggttgtttccaaaccctttttctatctagcctttttcagtctctcaacatttaagcagcaaaagaactcgagagagaaaacttgtactaaatatccttctttgaccggccctctcctctccccactacggggatttctgggtggctcacagtggacaaggaataggtaatcccaccaaaccttgaggtgggctaaactggagattttggtatgggtctcctactgtaaagagaaagccttccgggctaacggtattcctttcgcagtctactgcctcctttgtgaactaatgactgtaattattacctcccagagctcttttgttatcaacaacccggagccagaggggggtgggggatgggccctttgggaaaagggaaaaaaatttacaaagcaaattgctgtctacgaagggttggttttttaaaaagacaaacccaattccagcctgcattcgaagtggggagtggcaaaattttttttcaaagtatgataagattttaaaaatactcagagctgtgggattcaattgcatttccacagtatcgctttaagttactatttttgacgaagtaaaattcagatgttgaaaatctgtatctcttgttttcatccatttcttccttggaaggtgtgtgtgtgtgtgtgtgtgtgtgtgtgtgtgtgtgtgtgtgtgtgtgtgtgtgtttaagaaccttttttttttatttccgaccactcatccatggtaaaaagcttcaaccccagccagctggcttgaagagaattattttgcaggatttagtatggatttaaacaaagactcaggctctccaagtcttgttggcaaggctgggcggaagcgccctttccaggagctgttacctctgccagctgaagccaccaggcctggaggaccctaaagacttactaagttgaggcctagggtcaaggtgactgccttcccttagagacacgccttgggtagcacctcagcagtgccaatctcaccgccctccccctccccacctcgggccactcaccggacctcagtgggcatcctctagctagatcctccctggcccccctggattctggaaaccttgggaagaagataaagctttgtggagagaatgcacttggtcatctgcagttattcgaggtctccggatccctaacaaaataagtgatcctggtcaccaagactaaaggtcccagggtttctcctccggcaacagctttggtgactcatttgaaaaactcaaagaaggaataaaggactatggagagcagggaagctgcagtccctcgctcggagagaaggaaaggagatcgggaacggtttaaagcagcactttcctgcaagtctttcttgagctctctgtaagcctggaactatgggtttagtataggcaagaggaaacggaagcggagccagagggccccaaatcttcctcaaggcgccgtccctgcatttaagagcctttgggaaaagggaaacagaaaggattttttcattcctttattagaaaacacaaacgaaactacttctttctgggctgggaaattgccactgttgtgttcctaggcacctgctgatggcaagaactcctcttgggaagggacgaggtcagtgggttgagtatccctgaaaagatgggagtgccttttcctgggatttggaaaaactgattcgcttactttgagactccctgaatcctgtgtatgtgtcagctctcacccactccaagaagtttctgttcgttttatttatttaatttttctcagcctgaggtcctcagtgatagattccagcgtggattttaattgcttcaatcagcagcctttctcttcagccgtcagtcaaaacctggacgatgggtctggggacccaggcatgactgcacagaaaccgtacgacccccacccccaccccccaggctggctcagctcagcaggcagacattaggctctgctaaggagatgaaatgagttcgttggtgtggaagcggtccaccttcctccctccttggttccttccccaagctttggagctcttcctgattgaggccaggtggcctgggctcttgaggtcacagcgacctcagcactggtttggaggaaggcgggcgcgagaaccacttttgctcggcagcagccagagacagccctcaaacaatgagccaatcgatgcacacgtgaaattgccctcggccaccattccaatcttgccaaggtctccctgtccctggggtcacctaggccagcgtgctgagggctgtggtagcaccctggacagcgcgttccggcagaagcagacctggag

SEQ ID NO: 14 - DNA, 3000 bp, Mus musculus
  source 1..3000: mol_type = genomic DNA
tttccgttgagtggtgatgaaagtcgctaagatggtcacaaaaaaagagacaggcctgggataaaccatcgaagacccagaggtgcacatgaataaaccggtctgctgctccacaatatgagggaaatctctatgaaaacgagtaaagcgatcatagagtactccccatcactcagacaggcccaaaaatccagtttgttttgcccctaaaggatgagaaacggagggagaggaaaaagaaagccaggaggtagcggcgagaaggctagaagaggccggccgttacagagcctttcgggcatctccaggtgttgtctagggcgcaccagggaaaaggccgccagcacggggtctctgtgtgtttggcgccctctggtggaaattttttccaataccgcctttttatggtgggggacttcaccccgctcagtaatgtgcttaaatattgccaagagagaatcattgaacagcgtgaaactgaaaagaagcgaggagagcgggccaagacacggagtgccgtcctggcttcccggagccaccctccatgctctgctgccccaggcgtgtggagcggcactcgtgcgtgttattaaccttcagacatgatcaattacgaagatttcttttacccctctccagggagagggctcagagaaagggaaatagaccccttgcctcttgtggtgccaggtagctgtgttcgaacgaggtagtgtggagatggactggaagaagaaacgggagtgcagaaactccagggtctgtctgggtggtcccctcatctccgctttgcctgtacagccatactggctcagtagagcgctccctaggacaccacccagagaaaaccttctggaatcgccaatccaggacaaccacaggagattgatcaaggcaaagcaaatattctagtcttctccaagatacgggatggagggctaggaagaggggaaggaagaatcacccagtgagacaaaattcttcgtaggaattatattttcccttgccctcacccaacatcgcctatctcaaaaataatttaaaaacaaaaaacaaacaaacaaacaaaaaacagagcgtgctgagtgcattctggattactcataggactttgtcacacacaccctcctttctggtcgcaaacccgtgagctggatttataatcgccctacaaagctccagaggcagtcagacacctgcaaaggagccccagcgctccgcggacgagctgcccccgcgagcaacggcctcgtgattccccccgccgagcgggtccccgcctccccactccgcccccgcctcccccaagcccagcggccgcctctccggatctctcccttcttcaggctctcccgtgccggaccagggatcgtgcaagcaaggaagcagccctggggtgacacccagcacgtactcctgtgacagagccgagcccagcccagccccgggacgcttcgcagaggagtcgcgggagggtccagctcgctgtcgctgaaccgaggtgggtaaataccggatcgcccggacttgccagagccccgcctcggttattcaacccggtgccctcagcctgcggcttcttgtccagccctttgcctcaccccaccagcacgcgcctgtcgcccaccttccacagccgagtgcttcccgccagtcctgtcgcagctgtggtttggcgcacccatcccctaccctcctcgctcttgaaacccttatcaatttcattcgggaggacacataagggctgaagtgaccccagagccattttttgcctgcgcttgggggatcggagctcacggctgtcggatacgcgcctgggtagcagcggcagaaggtgcgaggagcgataacctgttacttccccagcacccgcgtcccaccgccgcccgcggagctgcgagagcgcgcggaggttgcggggggggggggggacagatgctcggcccgagggacgacacgcaaaaggcggctggtgggctgcgctctgcggggtcttagatttacccagattaccgttctcctccctctcctctcattctttcgcccgctccttctccccatctcttcctcttctctcgccctctctccctcactctgtccacgaacaaacaccaaataggggaaccgcgcactcttctatccgaggtctcttgcgccctaggcgcaaattcgccaccgggtgacggtctcctttttaccctctgccaccttctctggctcagtgaaacgaactctggggactaggtagagtagaaacagtgaatctgggacggagcctcgctctagggttgagaaagctagaaacgaggtgggacaagaaactgatcagcaaggcttcgacacgctgccttttggctgtctggagtgcaaggtgactgattcttagcgggtcaagtcctgaggggcggaggacctatttcttctcaccttgtctcaccaaagtccctgtccccggcgctgtgagcctccttctttccaaggaattggccagacacaacaacgggagccagacaccgaaccagacgtgcccgccccgcacgccctcccccctcctcttctgcccgttcaccaggctgctgggagcccaatggggcttgtctcggctgggctggaatttgctcgatgagtgctccctagtgctcctggccctatcctcaccccatccctcgcgtcctgcacccgcctccggcgccccttagctgtgagcctcactcggagcaccccgttgcgcctctagacttgagagtcgcccggggctactgtgcttgcgccccagtcccagagctagcgagcgcctccccaccccctcccaccgaccgcgcaccaggacccagccagctcgctgcccttggtctcccttctgtctccgagacttcggtgccccgggccgcaggacctagaagctctcccggcacagctctcccttctgtttgcagcctgttcctgcgcccagtctgcgggggacccttgaaccgtagagaccccaagaccaccgagctg

SEQ ID NO: 15 - DNA, 6687 bp, synthetic construct
  misc_feature 1..6687: note = pAAV mGAD65 (Ri-Rii-D-ETSS) GFP WPRE SV40pA
  misc_feature 2938: note = n is a, c, g, or t
  misc_feature 4209: note = n is a, c, g, or t
  source 1..6687: mol_type = other DNA
tcgagatttctgggtggctcacagtggacaaggaataggtaatcccaccaaaccttgaggtgggctaaactggagattttggtatgggtctcctactgtaaagagaaagccttccgggctaacggtattcctttcgcagtctactgcctcctttgtgaactaatgactgtaattattacctcccagagctcttttgttatcaacaacccggaggaaaagggaaacagaaaggattttttcattcctttattagaaaacacaaacgaaactacttctttctgggctgggaaattgccactgttgtgttcctaggcacctgctgatggcaagaactcctcttgggaagggacgaggtcagtgggttgagtatccctgaaaagatgggagtgccttttcctgggatttggaaaaactgattcgcttactttgagactccctgaatcctgtgtatgtgtcagctctcacccactccaagaagtttctgttcgttttatttatttaatttttctcagcctgaggtcctcagtgatagattccagcgtggattttaattgcttcaatcagcagcctttctcttcagccgtcagtcaaaacctggacgatgggtctggggacccaggcatgactgcacagaaaccgtacgacccccacccccaccccccaggctggctcagctcagcaggcagacattaggctctgctaaggagatgaaatgagttcgttggtgtggaagcggtccaccttcctccctccttggttccttccccaagctttggagctcttcctgattgaggccaggtggcctgggctcttgaggtcacagcgacctcagcactggtttggaggaaggcgggcgcgagaaccacttttgctcggcagcagccagagacagccctcaaacaatgagccaatcgatgcacacgtgaaattgccctcggccaccattccaatcttgccaaggtctccctgtccctggggtcacctaggccagcgtgctgagggctgtggtagcaccctggacagcgcgttccggcagaagcagacctggagcgcctgtggctgggtcagcactacgcaggcacgcctccctcccccgcatctgactcgcacctcacgacccagcgcctccatttcccttccgtcactctctcatctccccaccaagctccctcaccggtcgccaccatggtgagcaagggcgaggagctgttcaccggggtggtgcccatcctggtcgagctggacggcgacgtaaacggccacaagttcagcgtgtccggcgagggcgagggcgatgccacctacggcaagctgaccctgaagttcatctgcaccaccggcaagctgcccgtgccctggcccaccctcgtgaccaccctgacctacggcgtgcagtgcttcagccgctaccccgaccacatgaagcagcacgacttcttcaagtccgccatgcccgaaggctacgtccaggagcgcaccatcttcttcaaggacgacggcaactacaagacccgcgccgaggtgaagttcgagggcgacaccctggtgaaccgcatcgagctgaagggcatcgacttcaaggaggacggcaacatcctggggcacaagctggagtacaactacaacagccacaacgtctatatcatggccgacaagcagaagaacggcatcaaggtgaacttcaagatccgccacaacatcgaggacggcagcgtgcagctcgccgaccactaccagcagaacacccccatcggcgacggccccgtgctgctgcccgacaaccactacctgagcacccagtccgccctgagcaaagaccccaacgagaagcgcgatcacatggtcctgctggagttcgtgaccgccgccgggatcactctcggcatggacgagctgtacaagtaaagcggccgcatcgataatcaacctctggattacaaaatttgtgaaagattgactggtattcttaactatgttgctccttttacgctatgtggatacgctgctttaatgcctttgtatcatgctattgcttcccgtatggctttcattttctcctccttgtataaatcctggttgctgtctctttatgaggagttgtggcccgttgtcaggcaacgtggcgtggtgtgcactgtgtttgctgacgcaacccccactggttggggcattgccaccacctgtcagctcctttccgggactttcgctttccccctccctattgccacggcggaactcatcgccgcctgccttgcccgctgctggacaggggctcggctgttgggcactgacaattccgtggtgttgtcggggaagctgacgtcctttccatggctgctcgcctgtgttgccacctggattctgcgcgggacgtccttctgctacgtcccttcggccctcaatccagcggaccttccttcccgcggcctgctgccggctctgcggcctcttccgcgtcttcgccttcgccctcagacgagtcggatctccctttgggccgcctccccgcatcgatgccgtatacggtaccacttgtttattgcagcttataatggttacaaataaagcaatagcatcacaaatttcacaaataaagcatttttttcactgcattctagttgtggtttgtccaaactcatcaatgtatcttatcatgtctgtcgacccccaacgcgttggagctctagagcatggctacgtagataagtagcatggcgggttaatcattaactacaaggaacccctagtgatggagttggccactccctctctgcgcgctcgctcgctcactgaggccgggcgaccaaaggtcgcccgacgcccgggctttgcccgggcggcctcagtgagcgagcgagcgcgcagctggcgtaatagcgaagaggcccgcaccgatcgcccttcccaacagttgcgcagcctgaatggcgaatggaanttccaacatccaataaatcatacaggcaaggcaaagaattagcaaaattaagcaataaagcctcagagcataaagctaaatcggttgtaccaaaaacattatgaccctgtaatacttttgcgggagaagcctttatttcaacgcaaggataaaaatttttagaaccctcatatattttaaatgcaatgcctgagtaatgtgtaggtaaagattcaaacgggtgagaaaggccggagacagtcaaatcaccatcaatatgatattcaaccgttctagctgataaattcatgccggagagggtagctatttttgagaggtctctacaaaggctatcaggtcattgcctgagagtctggagcaaacaagagaatcgatgaacggtaatcgtaaaactagcatgtcaatcatatgtaccccggttgataatcagaaaagccccaaaaacaggaagattgtataagcaaatatttaaattgtaaacgttaatattttgttaaaattcgcgttaaatttttgttaaatcagctcattttttaaccaataggccgaaatcggcaaaatcccttataaatcaaaagaatagaccgagatagggttgagtgttgttccagtttggaacaagagtccactattaaagaacgtggactccaacgtcaaagggcgaaaaaccgtctatcagggcgatggcccactacgtgaaccatcaccctaatcaagttttttggggtcgaggtgccgtaaagcactaaatcggaaccctaaagggagcccccgatttagagcttgacggggaaagccggcgaacgtggcgagaaaggaagggaagaaagcgaaaggagcgggcgctagggcgctggcaagtgtagcggtcacgctgcgcgtaaccaccacacccgccgcgcttaatgcgccgctacagggcgcgtactatggttgctttgacgagcacgtataacgtgctttcctcgttagaatcagagcgggagctaaacaggaggccgattaaagggattttagacaggaacggtacgccagaatcctgagaagtgtttttataatcagtgaggccaccgagtaaaagagtctgtccatcacgcaaattaaccgttgtcgcaatacttctttgattagtaataacatcacttgcctgagtagaagaactcaaactatcggccttgctggtaatatccagaacaatattaccgccagccattgcaacaggaaaaacgctcatggaaatacctacattttgacgctcaatcgtctggaanttcctgatgcggtattttctccttacgcatctgtgcggtatttcacaccgcatatggtgcactctcagtacaatctgctctgatgccgcatagttaagccagccccgacacccgccaacacccgctgacgcgccctgacgggcttgtctgctcccggcatccgcttacagacaagctgtgaccgtctccgggagctgcatgtgtcagaggttttcaccgtcatcaccgaaacgcgcgagacgaaagggcctcgtgatacgcctatttttataggttaatgtcatgataataatggtttcttagacgtcaggtggcacttttcggggaaatgtgcgcggaacccctatttgtttatttttctaaatacattcaaatatgtatccgctcatgagacaataaccctgataaatgcttcaataatattgaaaaaggaagagtatgagtattcaacatttccgtgtcgcccttattcccttttttgcggcattttgccttcctgtttttgctcacccagaaacgctggtgaaagtaaaagatgctgaagatcagttgggtgcacgagtgggttacatcgaactggatctcaacagcggtaagatccttgagagttttcgccccgaagaacgttttccaatgatgagcacttttaaagttctgctatgtggcgcggtattatcccgtattgacgccgggcaagagcaactcggtcgccgcatacactattctcagaatgacttggttgagtactcaccagtcacagaaaagcatcttacggatggcatgacagtaagagaattatgcagtgctgccataaccatgagtgataacactgcggccaacttacttctgacaacgatcggaggaccgaaggagctaaccgcttttttgcacaacatgggggatcatgtaactcgccttgatcgttgggaaccggagctgaatgaagccataccaaacgacgagcgtgacaccacgatgcctgtagcaatggcaacaacgttgcgcaaactattaactggcgaactacttactctagcttcccggcaacaattaatagactggatggaggcggataaagttgcaggaccacttctgcgctcggcccttccggctggctggtttattgctgataaatctggagccggtgagcgtgggtctcgcggtatcattgcagcactggggccagatggtaagccctcccgtatcgtagttatctacacgacggggagtcaggcaactatggatgaacgaaatagacagatcgctgagataggtgcctcactgattaagcattggtaactgtcagaccaagtttactcatatatactttagattgatttaaaacttcatttttaatttaaaaggatctaggtgaagatcctttttgataatctcatgaccaaaatcccttaacgtgagttttcgttccactgagcgtcagaccccgtagaaaagatcaaaggatcttcttgagatcctttttttctgcgcgtaatctgctgcttgcaaacaaaaaaaccaccgctaccagcggtggtttgtttgccggatcaagagctaccaactctttttccgaaggtaactggcttcagcagagcgcagataccaaatactgtccttctagtgtagccgtagttaggccaccacttcaagaactctgtagcaccgcctacatacctcgctctgctaatcctgttaccagtggctgctgccagtggcgataagtcgtgtcttaccgggttggactcaagacgatagttaccggataaggcgcagcggtcgggctgaacggggggttcgtgcacacagcccagcttggagcgaacgacctacaccgaactgagatacctacagcgtgagctatgagaaagcgccacgcttcccgaagggagaaaggcggacaggtatccggtaagcggcagggtcggaacaggagagcgcacgagggagcttccagggggaaacgcctggtatctttatagtcctgtcgggtttcgccacctctgacttgagcgtcgatttttgtgatgctcgtcaggggggcggagcctatggaaaaacgccagcaacgcggcctttttacggttcctggccttttgctggccttttgctcacatgttctttcctgcgttatcccctgattctgtggataaccgtattaccgcctttgagtgagctgataccgctcgccgcagccgaacgaccgagcgcagcgagtcagtgagcgaggaagcggaagagcgcccaatacgcaaaccgcctctccccgcgcgttggccgattcattaatgcagctgcgcgctcgctcgctcactgaggccgcccgggcaaagcccgggcgtcgggcgacctttggtcgcccggcctcagtgagcgagcgagcgcgcagagagggagtggccaactccatcactaggggttccttgtagttaatgattaacccgccatgctacttatctacgtagccatgctctagac

SEQ ID NO: 16 - DNA, 6214 bp, synthetic construct
  misc_feature 1..6214: note = pAAV mGAD65 (Ri-Rii-ETSS) GFP WPRE SV40pA
  misc_feature 2465: note = n is a, c, g, or t
  misc_feature 3736: note = n is a, c, g, or t
  source 1..6214: mol_type = other DNA
tcgagatttctgggtggctcacagtggacaaggaataggtaatcccaccaaaccttgaggtgggctaaactggagattttggtatgggtctcctactgtaaagagaaagccttccgggctaacggtattcctttcgcagtctactgcctcctttgtgaactaatgactgtaattattacctcccagagctcttttgttatcaacaacccggaggaaaagggaaacagaaaggattttttcattcctttattagaaaacacaaacgaaactacttctttctgggctgggaaattgccactgttgtgttcctaggcacctgctgatggcaagaactcctcttgggaagggacgaggtcagtgggttgagtatccctgaaaagatgggagtgccttttcctgggatttggaaaaactgattcgcttactttgagactccctgaatcctgtgtatgtgtcagctctcacccactccaagaagtttctgttcgttttatttatttaatttttctcagcctgaggtcctcagtgatagattccagcgtggattttaattgcttcaatcagcagcctttctcttcgcctgtggctgggtcagcactacgcaggcacgcctccctcccccgcatctgactcgcacctcacgacccagcgcctccatttcccttccgtcactctctcatctccccaccaagctccctcaccggtcgccaccatggtgagcaagggcgaggagctgttcaccggggtggtgcccatcctggtcgagctggacggcgacgtaaacggccacaagttcagcgtgtccggcgagggcgagggcgatgccacctacggcaagctgaccctgaagttcatctgcaccaccggcaagctgcccgtgccctggcccaccctcgtgaccaccctgacctacggcgtgcagtgcttcagccgctaccccgaccacatgaagcagcacgacttcttcaagtccgccatgcccgaaggctacgtccaggagcgcaccatcttcttcaaggacgacggcaactacaagacccgcgccgaggtgaagttcgagggcgacaccctggtgaaccgcatcgagctgaagggcatcgacttcaaggaggacggcaacatcctggggcacaagctggagtacaactacaacagccacaacgtctatatcatggccgacaagcagaagaacggcatcaaggtgaacttcaagatccgccacaacatcgaggacggcagcgtgcagctcgccgaccactaccagcagaacacccccatcggcgacggccccgtgctgctgcccgacaaccactacctgagcacccagtccgccctgagcaaagaccccaacgagaagcgcgatcacatggtcctgctggagttcgtgaccgccgccgggatcactctcggcatggacgagctgtacaagtaaagcggccgcatcgataatcaacctctggattacaaaatttgtgaaagattgactggtattcttaactatgttgctccttttacgctatgtggatacgctgctttaatgcctttgtatcatgctattgcttcccgtatggctttcattttctcctccttgtataaatcctggttgctgtctctttatgaggagttgtggcccgttgtcaggcaacgtggcgtggtgtgcactgtgtttgctgacgcaacccccactggttggggcattgccaccacctgtcagctcctttccgggactttcgctttccccctccctattgccacggcggaactcatcgccgcctgccttgcccgctgctggacaggggctcggctgttgggcactgacaattccgtggtgttgtcggggaagctgacgtcctttccatggctgctcgcctgtgttgccacctggattctgcgcgggacgtccttctgctacgtcccttcggccctcaatccagcggaccttccttcccgcggcctgctgccggctctgcggcctcttccgcgtcttcgccttcgccctcagacgagtcggatctccctttgggccgcctccccgcatcgatgccgtatacggtaccacttgtttattgcagcttataatggttacaaataaagcaatagcatcacaaatttcacaaataaagcatttttttcactgcattctagttgtggtttgtccaaactcatcaatgtatcttatcatgtctgtcgacccccaacgcgttggagctctagagcatggctacgtagataagtagcatggcgggttaatcattaactacaaggaacccctagtgatggagttggccactccctctctgcgcgctcgctcgctcactgaggccgggcgaccaaaggtcgcccgacgcccgggctttgcccgggcggcctcagtgagcgagcgagcgcgcagctggcgtaatagcgaagaggcccgcaccgatcgcccttcccaacagttgcgcagcctgaatggcgaatggaanttccaacatccaataaatcatacaggcaaggcaaagaattagcaaaattaagcaataaagcctcagagcataaagctaaatcggttgtaccaaaaacattatgaccctgtaatacttttgcgggagaagcctttatttcaacgcaaggataaaaatttttagaaccctcatatattttaaatgcaatgcctgagtaatgtgtaggtaaagattcaaacgggtgagaaaggccggagacagtcaaatcaccatcaatatgatattcaaccgttctagctgataaattcatgccggagagggtagctatttttgagaggtctctacaaaggctatcaggtcattgcctgagagtctggagcaaacaagagaatcgatgaacggtaatcgtaaaactagcatgtcaatcatatgtaccccggttgataatcagaaaagccccaaaaacaggaagattgtataagcaaatatttaaattgtaaacgttaatattttgttaaaattcgcgttaaatttttgttaaatcagctcattttttaaccaataggccgaaatcggcaaaatcccttataaatcaaaagaatagaccgagatagggttgagtgttgttccagtttggaacaagagtccactattaaagaacgtggactccaacgtcaaagggcgaaaaaccgtctatcagggcgatggcccactacgtgaaccatcaccctaatcaagttttttggggtcgaggtgccgtaaagcactaaatcggaaccctaaagggagcccccgatttagagcttgacggggaaagccggcgaacgtggcgagaaaggaagggaagaaagcgaaaggagcgggcgctagggcgctggcaagtgtagcggtcacgctgcgcgtaaccaccacacccgccgcgcttaatgcgccgctacagggcgcgtactatggttgctttgacgagcacgtataacgtgctttcctcgttagaatcagagcgggagctaaacaggaggccgattaaagggattttagacaggaacggtacgccagaatcctgagaagtgtttttataatcagtgaggccaccgagtaaaagagtctgtccatcacgcaaattaaccgttgtcgcaatacttctttgattagtaataacatcacttgcctgagtagaagaactcaaactatcggccttgctggtaatatccagaacaatattaccgccagccattgcaacaggaaaaacgctcatggaaatacctacattttgacgctcaatcgtctggaanttcctgatgcggtattttctccttacgcatctgtgcggtatttcacaccgcatatggtgcactctcagtacaatctgctctgatgccgcatagttaagccagccccgacacccgccaacacccgctgacgcgccctgacgggcttgtctgctcccggcatccgcttacagacaagctgtgaccgtctccgggagctgcatgtgtcagaggttttcaccgtcatcaccgaaacgcgcgagacgaaagggcctcgtgatacgcctatttttataggttaatgtcatgataataatggtttcttagacgtcaggtggcacttttcggggaaatgtgcgcggaacccctatttgtttatttttctaaatacattcaaatatgtatccgctcatgagacaataaccctgataaatgcttcaataatattgaaaaaggaagagtatgagtattcaacatttccgtgtcgcccttattcccttttttgcggcattttgccttcctgtttttgctcacccagaaacgctggtgaaagtaaaagatgctgaagatcagttgggtgcacgagtgggttacatcgaactggatctcaacagcggtaagatccttgagagttttcgccccgaagaacgttttccaatgatgagcacttttaaagttctgctatgtggcgcggtattatcccgtattgacgccgggcaagagcaactcggtcgccgcatacactattctcagaatgacttggttgagtactcaccagtcacagaaaagcatcttacggatggcatgacagtaagagaattatgcagtgctgccataaccatgagtgataacactgcggccaacttacttctgacaacgatcggaggaccgaaggagctaaccgcttttttgcacaacatgggggatcatgtaactcgccttgatcgttgggaaccggagctgaatgaagccataccaaacgacgagcgtgacaccacgatgcctgtagcaatggcaacaacgttgcgcaaactattaactggcgaactacttactctagcttcccggcaacaattaatagactggatggaggcggataaagttgcaggaccacttctgcgctcggcccttccggctggctggtttattgctgataaatctggagccggtgagcgtgggtctcgcggtatcattgcagcactggggccagatggtaagccctcccgtatcgtagttatctacacgacggggagtcaggcaactatggatgaacgaaatagacagatcgctgagataggtgcctcactgattaagcattggtaactgtcagaccaagtttactcatatatactttagattgatttaaaacttcatttttaatttaaaaggatctaggtgaagatcctttttgataatctcatgaccaaaatcccttaacgtgagttttcgttccactgagcgtcagaccccgtagaaaagatcaaaggatcttcttgagatcctttttttctgcgcgtaatctgctgcttgcaaacaaaaaaaccaccgctaccagcggtggtttgtttgccggatcaagagctaccaactctttttccgaaggtaactggcttcagcagagcgcagataccaaatactgtccttctagtgtagccgtagttaggccaccacttcaagaactctgtagcaccgcctacatacctcgctctgctaatcctgttaccagtggctgctgccagtggcgataagtcgtgtcttaccgggttggactcaagacgatagttaccggataaggcgcagcggtcgggctgaacggggggttcgtgcacacagcccagcttggagcgaacgacctacaccgaactgagatacctacagcgtgagctatgagaaagcgccacgcttcccgaagggagaaaggcggacaggtatccggtaagcggcagggtcggaacaggagagcgcacgagggagcttccagggggaaacgcctggtatctttatagtcctgtcgggtttcgccacctctgacttgagcgtcgatttttgtgatgctcgtcaggggggcggagcctatggaaaaacgccagcaacgcggcctttttacggttcctggccttttgctggccttttgctcacatgttctttcctgcgttatcccctgattctgtggataaccgtattaccgcctttgagtgagctgataccgctcgccgcagccgaacgaccgagcgcagcgagtcagtgagcgaggaagcggaagagcgcccaatacgcaaaccgcctctccccgcgcgttggccgattcattaatgcagctgcgcgctcgctcgctcactgaggccgcccgggcaaagcccgggcgtcgggcgacctttggtcgcccggcctcagtgagcgagcgagcgcgcagagagggagtggccaactccatcactaggggttccttgtagttaatgattaacccgccatgctacttatctacgtagccatgctctagac

SEQ ID NO: 17 - DNA, 6006 bp, synthetic construct
  misc_feature 1..6006: note = pAAV mGAD65 (Rii-ETSS) GFP WPRE SV40pA
  misc_feature 2257: note = n is a, c, g, or t
  misc_feature 3528: note = n is a, c, g, or t
  source 1..6006: mol_type = other DNA
tcgaggaaaagggaaacagaaaggattttttcattcctttattagaaaacacaaacgaaactacttctttctgggctgggaaattgccactgttgtgttcctaggcacctgctgatggcaagaactcctcttgggaagggacgaggtcagtgggttgagtatccctgaaaagatgggagtgccttttcctgggatttggaaaaactgattcgcttactttgagactccctgaatcctgtgtatgtgtcagctctcacccactccaagaagtttctgttcgttttatttatttaatttttctcagcctgaggtcctcagtgatagattccagcgtggattttaattgcttcaatcagcagcctttctcttcgcctgtggctgggtcagcactacgcaggcacgcctccctcccccgcatctgactcgcacctcacgacccagcgcctccatttcccttccgtcactctctcatctccccaccaagctccctcaccggtcgccaccatggtgagcaagggcgaggagctgttcaccggggtggtgcccatcctggtcgagctggacggcgacgtaaacggccacaagttcagcgtgtccggcgagggcgagggcgatgccacctacggcaagctgaccctgaagttcatctgcaccaccggcaagctgcccgtgccctggcccaccctcgtgaccaccctgacctacggcgtgcagtgcttcagccgctaccccgaccacatgaagcagcacgacttcttcaagtccgccatgcccgaaggctacgtccaggagcgcaccatcttcttcaaggacgacggcaactacaagacccgcgccgaggtgaagttcgagggcgacaccctggtgaaccgcatcgagctgaagggcatcgacttcaaggaggacggcaacatcctggggcacaagctggagtacaactacaacagccacaacgtctatatcatggccgacaagcagaagaacggcatcaaggtgaacttcaagatccgccacaacatcgaggacggcagcgtgcagctcgccgaccactaccagcagaacacccccatcggcgacggccccgtgctgctgcccgacaaccactacctgagcacccagtccgccctgagcaaagaccccaacgagaagcgcgatcacatggtcctgctggagttcgtgaccgccgccgggatcactctcggcatggacgagctgtacaagtaaagcggccgcatcgataatcaacctctggattacaaaatttgtgaaagattgactggtattcttaactatgttgctccttttacgctatgtggatacgctgctttaatgcctttgtatcatgctattgcttcccgtatggctttcattttctcctccttgtataaatcctggttgctgtctctttatgaggagttgtggcccgttgtcaggcaacgtggcgtggtgtgcactgtgtttgctgacgcaacccccactggttggggcattgccaccacctgtcagctcctttccgggactttcgctttccccctccctattgccacggcggaactcatcgccgcctgccttgcccgctgctggacaggggctcggctgttgggcactgacaattccgtggtgttgtcggggaagctgacgtcctttccatggctgctcgcctgtgttgccacctggattctgcgcgggacgtccttctgctacgtcccttcggccctcaatccagcggaccttccttcccgcggcctgctgccggctctgcggcctcttccgcgtcttcgccttcgccctcagacgagtcggatctccctttgggccgcctccccgcatcgatgccgtatacggtaccacttgtttattgcagcttataatggttacaaataaagcaatagcatcacaaatttcacaaataaagcatttttttcactgcattctagttgtggtttgtccaaactcatcaatgtatcttatcatgtctgtcgacccccaacgcgttggagctctagagcatggctacgtagataagtagcatggcgggttaatcattaactacaaggaacccctagtgatggagttggccactccctctctgcgcgctcgctcgctcactgaggccgggcgaccaaaggtcgcccgacgcccgggctttgcccgggcggcctcagtgagcgagcgagcgcgcagctggcgtaatagcgaagaggcccgcaccgatcgcccttcccaacagttgcgcagcctgaatggcgaatggaanttccaacatccaataaatcatacaggcaaggcaaagaattagcaaaattaagcaataaagcctcagagcataaagctaaatcggttgtaccaaaaacattatgaccctgtaatacttttgcgggagaagcctttatttcaacgcaaggataaaaatttttagaaccctcatatattttaaatgcaatgcctgagtaatgtgtaggtaaagattcaaacgggtgagaaaggccggagacagtcaaatcaccatcaatatgatattcaaccgttctagctgataaattcatgccggagagggtagctatttttgagaggtctctacaaaggctatcaggtcattgcctgagagtctggagcaaacaagagaatcgatgaacggtaatcgtaaaactagcatgtcaatcatatgtaccccggttgataatcagaaaagccccaaaaacaggaagattgtataagcaaatatttaaattgtaaacgttaatattttgttaaaattcgcgttaaatttttgttaaatcagctcattttttaaccaataggccgaaatcggcaaaatcccttataaatcaaaagaatagaccgagatagggttgagtgttgttccagtttggaacaagagtccactattaaagaacgtggactccaacgtcaaagggcgaaaaaccgtctatcagggcgatggcccactacgtgaaccatcaccctaatcaagttttttggggtcgaggtgccgtaaagcactaaatcggaaccctaaagggagcccccgatttagagcttgacggggaaagccggcgaacgtggcgagaaaggaagggaagaaagcgaaaggagcgggcgctagggcgctggcaagtgtagcggtcacgctgcgcgtaaccaccacacccgccgcgcttaatgcgccgctacagggcgcgtactatggttgctttgacgagcacgtataacgtgctttcctcgttagaatcagagcgggagctaaacaggaggccgattaaagggattttagacaggaacggtacgccagaatcctgagaagtgtttttataatcagtgaggccaccgagtaaaagagtctgtccatcacgcaaattaaccgttgtcgcaatacttctttgattagtaataacatcacttgcctgagtagaagaactcaaactatcggccttgctggtaatatccagaacaatattaccgccagccattgcaacaggaaaaacgctcatggaaatacctacattttgacgctcaatcgtctggaanttcctgatgcggtattttctccttacgcatctgtgcggtatttcacaccgcatatggtgcactctcagtacaatctgctctgatgccgcatagttaagccagccccgacacccgccaacacccgctgacgcgccctgacgggcttgtctgctcccggcatccgcttacagacaagctgtgaccgtctccgggagctgcatgtgtcagaggttttcaccgtcatcaccgaaacgcgcgagacgaaagggcctcgtgatacgcctatttttataggttaatgtcatgataataatggtttcttagacgtcaggtggcacttttcggggaaatgtgcgcggaacccctatttgtttatttttctaaatacattcaaatatgtatccgctcatgagacaataaccctgataaatgcttcaataatattgaaaaaggaagagtatgagtattcaacatttccgtgtcgcccttattcccttttttgcggcattttgccttcctgtttttgctcacccagaaacgctggtgaaagtaaaagatgctgaagatcagttgggtgcacgagtgggttacatcgaactggatctcaacagcggtaagatccttgagagttttcgccccgaagaacgttttccaatgatgagcacttttaaagttctgctatgtggcgcggtattatcccgtattgacgccgggcaagagcaactcggtcgccgcatacactattctcagaatgacttggttgagtactcaccagtcacagaaaagcatcttacggatggcatgacagtaagagaattatgcagtgctgccataaccatgagtgataacactgcggccaacttacttctgacaacgatcggaggaccgaaggagctaaccgcttttttgcacaacatgggggatcatgtaactcgccttgatcgttgggaaccggagctgaatgaagccataccaaacgacgagcgtgacaccacgatgcctgtagcaatggcaacaacgttgcgcaaactattaactggcgaactacttactctagcttcccggcaacaattaatagactggatggaggcggataaagttgcaggaccacttctgcgctcggcccttccggctggctggtttattgctgataaatctggagccggtgagcgtgggtctcgcggtatcattgcagcactggggccagatggtaagccctcccgtatcgtagttatctacacgacggggagtcaggcaactatggatgaacgaaatagacagatcgctgagataggtgcctcactgattaagcattggtaactgtcagaccaagtttactcatatatactttagattgatttaaaacttcatttttaatttaaaaggatctaggtgaagatcctttttgataatctcatgaccaaaatcccttaacgtgagttttcgttccactgagcgtcagaccccgtagaaaagatcaaaggatcttcttgagatcctttttttctgcgcgtaatctgctgcttgcaaacaaaaaaaccaccgctaccagcggtggtttgtttgccggatcaagagctaccaactctttttccgaaggtaactggcttcagcagagcgcagataccaaatactgtccttctagtgtagccgtagttaggccaccacttcaagaactctgtagcaccgcctacatacctcgctctgctaatcctgttaccagtggctgctgccagtggcgataagtcgtgtcttaccgggttggactcaagacgatagttaccggataaggcgcagcggtcgggctgaacggggggttcgtgcacacagcccagcttggagcgaacgacctacaccgaactgagatacctacagcgtgagctatgagaaagcgccacgcttcccgaagggagaaaggcggacaggtatccggtaagcggcagggtcggaacaggagagcgcacgagggagcttccagggggaaacgcctggtatctttatagtcctgtcgggtttcgccacctctgacttgagcgtcgatttttgtgatgctcgtcaggggggcggagcctatggaaaaacgccagcaacgcggcctttttacggttcctggccttttgctggccttttgctcacatgttctttcctgcgttatcccctgattctgtggataaccgtattaccgcctttgagtgagctgataccgctcgccgcagccgaacgaccgagcgcagcgagtcagtgagcgaggaagcggaagagcgcccaatacgcaaaccgcctctccccgcgcgttggccgattcattaatgcagctgcgcgctcgctcgctcactgaggccgcccgggcaaagcccgggcgtcgggcgacctttggtcgcccggcctcagtgagcgagcgagcgcgcagagagggagtggccaactccatcactaggggttccttgtagttaatgattaacccgccatgctacttatctacgtagccatgctctagac

SEQ ID NO: 18 - DNA, 6487 bp, synthetic construct
  misc_feature 1..6487: note = pAAV mGAD67 (Ri-M-Rii-ETSS) GFP WPRE SV40pA
  misc_feature 2738: note = n is a, c, g, or t
  misc_feature 4009: note = n is a, c, g, or t
  source 1..6487: mol_type = other DNA
tcgagcttcaccccgctcagtaatgtgcttaaatattgccaagagagaatcattgaacagcgtgaaactgaaaagaagcgaggagagcgggccaagacacggagtgccgtcctggcttcccggagccaccctccatgctctgctgccccaggcgtgtggagcggcactcgtgcgtgttattaaccttcagacatgatcaattacgaagatttcttttacccctctccagggagagggctcagagaaagggaaatagaccccttgcctcttgtggtgccaggtagctgtgttcgaacgaggtagtgtggagatggactggaagaagaaacgggagtgcagaaactccagggtctgtctgggtggtcccctcatctccgctttgcctgtacagccatactggctcagtagagcgctccctaggacaccacccagagaaaaccttctggaatcgccaatccaggacaaccacaggagattgatcaaggcaaagcaaatattctagtcttctccaagatacgggatggagggctaggaagaggggaaggaagaatcacccagtgagacaaaattcttcgtaggaattatattttcccttgccctcacccaacatcgcctatctcaaaaataatttaaaaacaaaaaacaaacaaacaaacaaaaaacagagcgtgctgagtgcattctggattactcataggactttgtcacacacaccctcctttctggtcgcaaacccgtgagctggatttataatcgccctacaaagctccagaggcagtcagacacctgcaaaggagccccagcgctccgcggacgagctgcccccgcgagcaacggcctcgtgattccccccgccgagcgggtccccgcctccccactccgcccccgcctcccccaagcccagcggccgcctctccggatctctcccttcttcaggctctcccgtgccggaccagggatcgtgcaagcaagaccggtcgccaccatggtgagcaagggcgaggagctgttcaccggggtggtgcccatcctggtcgagctggacggcgacgtaaacggccacaagttcagcgtgtccggcgagggcgagggcgatgccacctacggcaagctgaccctgaagttcatctgcaccaccggcaagctgcccgtgccctggcccaccctcgtgaccaccctgacctacggcgtgcagtgcttcagccgctaccccgaccacatgaagcagcacgacttcttcaagtccgccatgcccgaaggctacgtccaggagcgcaccatcttcttcaaggacgacggcaactacaagacccgcgccgaggtgaagttcgagggcgacaccctggtgaaccgcatcgagctgaagggcatcgacttcaaggaggacggcaacatcctggggcacaagctggagtacaactacaacagccacaacgtctatatcatggccgacaagcagaagaacggcatcaaggtgaacttcaagatccgccacaacatcgaggacggcagcgtgcagctcgccgaccactaccagcagaacacccccatcggcgacggccccgtgctgctgcccgacaaccactacctgagcacccagtccgccctgagcaaagaccccaacgagaagcgcgatcacatggtcctgctggagttcgtgaccgccgccgggatcactctcggcatggacgagctgtacaagtaaagcggccgcatcgataatcaacctctggattacaaaatttgtgaaagattgactggtattcttaactatgttgctccttttacgctatgtggatacgctgctttaatgcctttgtatcatgctattgcttcccgtatggctttcattttctcctccttgtataaatcctggttgctgtctctttatgaggagttgtggcccgttgtcaggcaacgtggcgtggtgtgcactgtgtttgctgacgcaacccccactggttggggcattgccaccacctgtcagctcctttccgggactttcgctttccccctccctattgccacggcggaactcatcgccgcctgccttgcccgctgctggacaggggctcggctgttgggcactgacaattccgtggtgttgtcggggaagctgacgtcctttccatggctgctcgcctgtgttgccacctggattctgcgcgggacgtccttctgctacgtcccttcggccctcaatccagcggaccttccttcccgcggcctgctgccggctctgcggcctcttccgcgtcttcgccttcgccctcagacgagtcggatctccctttgggccgcctccccgcatcgatgccgtatacggtaccacttgtttattgcagcttataatggttacaaataaagcaatagcatcacaaatttcacaaataaagcatttttttcactgcattctagttgtggtttgtccaaactcatcaatgtatcttatcatgtctgtcgacccccaacgcgttggagctctagagcatggctacgtagataagtagcatggcgggttaatcattaactacaaggaacccctagtgatggagttggccactccctctctgcgcgctcgctcgctcactgaggccgggcgaccaaaggtcgcccgacgcccgggctttgcccgggcggcctcagtgagcgagcgagcgcgcagctggcgtaatagcgaagaggcccgcaccgatcgcccttcccaacagttgcgcagcctgaatggcgaatggaanttccaacatccaataaatcatacaggcaaggcaaagaattagcaaaattaagcaataaagcctcagagcataaagctaaatcggttgtaccaaaaacattatgaccctgtaatacttttgcgggagaagcctttatttcaacgcaaggataaaaatttttagaaccctcatatattttaaatgcaatgcctgagtaatgtgtaggtaaagattcaaacgggtgagaaaggccggagacagtcaaatcaccatcaatatgatattcaaccgttctagctgataaattcatgccggagagggtagctatttttgagaggtctctacaaaggctatcaggtcattgcctgagagtctggagcaaacaagagaatcgatgaacggtaatcgtaaaactagcatgtcaatcatatgtaccccggttgataatcagaaaagccccaaaaacaggaagattgtataagcaaatatttaaattgtaaacgttaatattttgttaaaattcgcgttaaatttttgttaaatcagctcattttttaaccaataggccgaaatcggcaaaatcccttataaatcaaaagaatagaccgagatagggttgagtgttgttccagtttggaacaagagtccactattaaagaacgtggactccaacgtcaaagggcgaaaaaccgtctatcagggcgatggcccactacgtgaaccatcaccctaatcaagttttttggggtcgaggtgccgtaaagcactaaatcggaaccctaaagggagcccccgatttagagcttgacggggaaagccggcgaacgtggcgagaaaggaagggaagaaagcgaaaggagcgggcgctagggcgctggcaagtgtagcggtcacgctgcgcgtaaccaccacacccgccgcgcttaatgcgccgctacagggcgcgtactatggttgctttgacgagcacgtataacgtgctttcctcgttagaatcagagcgggagctaaacaggaggccgattaaagggattttagacaggaacggtacgccagaatcctgagaagtgtttttataatcagtgaggccaccgagtaaaagagtctgtccatcacgcaaattaaccgttgtcgcaatacttctttgattagtaataacatcacttgcctgagtagaagaactcaaactatcggccttgctggtaatatccagaacaatattaccgccagccattgcaacaggaaaaacgctcatggaaatacctacattttgacgctcaatcgtctggaanttcctgatgcggtattttctccttacgcatctgtgcggtatttcacaccgcatatggtgcactctcagtacaatctgctctgatgccgcatagttaagccagccccgacacccgccaacacccgctgacgcgccctgacgggcttgtctgctcccggcatccgcttacagacaagctgtgaccgtctccgggagctgcatgtgtcagaggttttcaccgtcatcaccgaaacgcgcgagacgaaagggcctcgtgatacgcctatttttataggttaatgtcatgataataatggtttcttagacgtcaggtggcacttttcggggaaatgtgcgcggaacccctatttgtttatttttctaaatacattcaaatatgtatccgctcatgagacaataaccctgataaatgcttcaataatattgaaaaaggaagagtatgagtattcaacatttccgtgtcgcccttattcccttttttgcggcattttgccttcctgtttttgctcacccagaaacgctggtgaaagtaaaagatgctgaagatcagttgggtgcacgagtgggttacatcgaactggatctcaacagcggtaagatccttgagagttttcgccccgaagaacgttttccaatgatgagcacttttaaagttctgctatgtggcgcggtattatcccgtattgacgccgggcaagagcaactcggtcgccgcatacactattctcagaatgacttggttgagtactcaccagtcacagaaaagcatcttacggatggcatgacagtaagagaattatgcagtgctgccataaccatgagtgataacactgcggccaacttacttctgacaacgatcggaggaccgaaggagctaaccgcttttttgcacaacatgggggatcatgtaactcgccttgatcgttgggaaccggagctgaatgaagccataccaaacgacgagcgtgacaccacgatgcctgtagcaatggcaacaacgttgcgcaaactattaactggcgaactacttactctagcttcccggcaacaattaatagactggatggaggcggataaagttgcaggaccacttctgcgctcggcccttccggctggctggtttattgctgataaatctggagccggtgagcgtgggtctcgcggtatcattgcagcactggggccagatggtaagccctcccgtatcgtagttatctacacgacggggagtcaggcaactatggatgaacgaaatagacagatcgctgagataggtgcctcactgattaagcattggtaactgtcagaccaagtttactcatatatactttagattgatttaaaacttcatttttaatttaaaaggatctaggtgaagatcctttttgataatctcatgaccaaaatcccttaacgtgagttttcgttccactgagcgtcagaccccgtagaaaagatcaaaggatcttcttgagatcctttttttctgcgcgtaatctgctgcttgcaaacaaaaaaaccaccgctaccagcggtggtttgtttgccggatcaagagctaccaactctttttccgaaggtaactggcttcagcagagcgcagataccaaatactgtccttctagtgtagccgtagttaggccaccacttcaagaactctgtagcaccgcctacatacctcgctctgctaatcctgttaccagtggctgctgccagtggcgataagtcgtgtcttaccgggttggactcaagacgatagttaccggataaggcgcagcggtcgggctgaacggggggttcgtgcacacagcccagcttggagcgaacgacctacaccgaactgagatacctacagcgtgagctatgagaaagcgccacgcttcccgaagggagaaaggcggacaggtatccggtaagcggcagggtcggaacaggagagcgcacgagggagcttccagggggaaacgcctggtatctttatagtcctgtcgggtttcgccacctctgacttgagcgtcgatttttgtgatgctcgtcaggggggcggagcctatggaaaaacgccagcaacgcggcctttttacggttcctggccttttgctggccttttgctcacatgttctttcctgcgttatcccctgattctgtggataaccgtattaccgcctttgagtgagctgataccgctcgccgcagccgaacgaccgagcgcagcgagtcagtgagcgaggaagcggaagagcgcccaatacgcaaaccgcctctccccgcgcgttggccgattcattaatgcagctgcgcgctcgctcgctcactgaggccgcccgggcaaagcccgggcgtcgggcgacctttggtcgcccggcctcagtgagcgagcgagcgcgcagagagggagtggccaactccatcactaggggttccttgtagttaatgattaacccgccatgctacttatctacgtagccatgctctagac

SEQ ID NO: 19 - DNA, 6208 bp, synthetic construct
  misc_feature 1..6208: note = pAAV mGAD67 (Ri-Rii-ETSS) GFP WPRE SV40pA
  misc_feature 2459: note = n is a, c, g, or t
  misc_feature 3730: note = n is a, c, g, or t
  source 1..6208: mol_type = other DNA
tcgagcttcaccccgctcagtaatgtgcttaaatattgccaagagagaatcattgaacagcgtgaaactgaaaagaagcgaggagagcgggccaagacacggagtgccgtcctggcttcccggagccaccctccatgctctgctgccccaggcgtgtggagcggcactcgtgcgtgttattaaccttcagacatgatcaattacgaagatttcttttacccctctccagggagagggctcagagaaagggaaatagaccccttgcctcttgtggtgccaggtgacaaaattcttcgtaggaattatattttcccttgccctcacccaacatcgcctatctcaaaaataatttaaaaacaaaaaacaaacaaacaaacaaaaaacagagcgtgctgagtgcattctggattactcataggactttgtcacacacaccctcctttctggtcgcaaacccgtgagctggatttataatcgccctacaaagctccagaggcagtcagacacctgcaaaggagccccagcgctccgcggacgagctgcccccgcgagcaacggcctcgtgattccccccgccgagcgggtccccgcctccccactccgcccccgcctcccccaagcccagcggccgcctctccggatctctcccttcttcaggctctcccgtgccggaccagggatcgtgcaagcaagaccggtcgccaccatggtgagcaagggcgaggagctgttcaccggggtggtgcccatcctggtcgagctggacggcgacgtaaacggccacaagttcagcgtgtccggcgagggcgagggcgatgccacctacggcaagctgaccctgaagttcatctgcaccaccggcaagctgcccgtgccctggcccaccctcgtgaccaccctgacctacggcgtgcagtgcttcagccgctaccccgaccacatgaagcagcacgacttcttcaagtccgccatgcccgaaggctacgtccaggagcgcaccatcttcttcaaggacgacggcaactacaagacccgcgccgaggtgaagttcgagggcgacaccctggtgaaccgcatcgagctgaagggcatcgacttcaaggaggacggcaacatcctggggcacaagctggagtacaactacaacagccacaacgtctatatcatggccgacaagcagaagaacggcatcaaggtgaacttcaagatccgccacaacatcgaggacggcagcgtgcagctcgccgaccactaccagcagaacacccccatcggcgacggccccgtgctgctgcccgacaaccactacctgagcacccagtccgccctgagcaaagaccccaacgagaagcgcgatcacatggtcctgctggagttcgtgaccgccgccgggatcactctcggcatggacgagctgtacaagtaaagcggccgcatcgataatcaacctctggattacaaaatttgtgaaagattgactggtattcttaactatgttgctccttttacgctatgtggatacgctgctttaatgcctttgtatcatgctattgcttcccgtatggctttcattttctcctccttgtataaatcctggttgctgtctctttatgaggagttgtggcccgttgtcaggcaacgtggcgtggtgtgcactgtgtttgctgacgcaacccccactggttggggcattgccaccacctgtcagctcctttccgggactttcgctttccccctccctattgccacggcggaactcatcgccgcctgccttgcccgctgctggacaggggctcggctgttgggcactgacaattccgtggtgttgtcggggaagctgacgtcctttccatggctgctcgcctgtgttgccacctggattctgcgcgggacgtccttctgctacgtcccttcggccctcaatccagcggaccttccttcccgcggcctgctgccggctctgcggcctcttccgcgtcttcgccttcgccctcagacgagtcggatctccctttgggccgcctccccgcatcgatgccgtatacggtaccacttgtttattgcagcttataatggttacaaataaagcaatagcatcacaaatttcacaaataaagcatttttttcactgcattctagttgtggtttgtccaaactcatcaatgtatcttatcatgtctgtcgacccccaacgcgttggagctctagagcatggctacgtagataagtagcatggcgggttaatcattaactacaaggaacccctagtgatggagttggccactccctctctgcgcgctcgctcgctcactgaggccgggcgaccaaaggtcgcccgacgcccgggctttgcccgggcggcctcagtgagcgagcgagcgcgcagctggcgtaatagcgaagaggcccgcaccgatcgcccttcccaacagttgcgcagcctgaatggcgaatggaanttccaacatccaataaatcatacaggcaaggcaaagaattagcaaaattaagcaataaagcctcagagcataaagctaaatcggttgtaccaaaaacattatgaccctgtaatacttttgcgggagaagcctttatttcaacgcaaggataaaaatttttagaaccctcatatattttaaatgcaatgcctgagtaatgtgtaggtaaagattcaaacgggtgagaaaggccggagacagtcaaatcaccatcaatatgatattcaaccgttctagctgataaattcatgccggagagggtagctatttttgagaggtctctacaaaggctatcaggtcattgcctgagagtctggagcaaacaagagaatcgatgaacggtaatcgtaaaactagcatgtcaatcatatgtaccccggttgataatcagaaaagccccaaaaacaggaagattgtataagcaaatatttaaattgtaaacgttaatattttgttaaaattcgcgttaaatttttgttaaatcagctcattttttaaccaataggccgaaatcggcaaaatcccttataaatcaaaagaatagaccgagatagggttgagtgttgttccagtttggaacaagagtccactattaaagaacgtggactccaacgtcaaagggcgaaaaaccgtctatcagggcgatggcccactacgtgaaccatcaccctaatcaagttttttggggtcgaggtgccgtaaagcactaaatcggaaccctaaagggagcccccgatttagagcttgacggggaaagccggcgaacgtggcgagaaaggaagggaagaaagcgaaaggagcgggcgctagggcgctggcaagtgtagcggtcacgctgcgcgtaaccaccacacccgccgcgcttaatgcgccgctacagggcgcgtactatggttgctttgacgagcacgtataacgtgctttcctcgttagaatcagagcgggagctaaacaggaggccgattaaagggattttagacaggaacggtacgccagaatcctgagaagtgtttttataatcagtgaggccaccgagtaaaagagtctgtccatcacgcaaattaaccgttgtcgcaatacttctttgattagtaataacatcacttgcctgagtagaagaactcaaactatcggccttgctggtaatatccagaacaatattaccgccagccattgcaacaggaaaaacgctcatggaaatacctacattttgacgctcaatcgtctggaanttcctgatgcggtattttctccttacgcatctgtgcggtatttcacaccgcatatggtgcactctcagtacaatctgctctgatgccgcatagttaagccagccccgacacccgccaacacccgctgacgcgccctgacgggcttgtctgctcccggcatccgcttacagacaagctgtgaccgtctccgggagctgcatgtgtcagaggttttcaccgtcatcaccgaaacgcgcgagacgaaagggcctcgtgatacgcctatttttataggttaatgtcatgataataatggtttcttagacgtcaggtggcacttttcggggaaatgtgcgcggaacccctatttgtttatttttctaaatacattcaaatatgtatccgctcatgagacaataaccctgataaatgcttcaataatattgaaaaaggaagagtatgagtattcaacatttccgtgtcgcccttattcccttttttgcggcattttgccttcctgtttttgctcacccagaaacgctggtgaaagtaaaagatgctgaagatcagttgggtgcacgagtgggttacatcgaactggatctcaacagcggtaagatccttgagagttttcgccccgaagaacgttttccaatgatgagcacttttaaagttctgctatgtggcgcggtattatcccgtattgacgccgggcaagagcaactcggtcgccgcatacactattctcagaatgacttggttgagtactcaccagtcacagaaaagcatcttacggatggcatgacagtaagagaattatgcagtgctgccataaccatgagtgataacactgcggccaacttacttctgacaacgatcggaggaccgaaggagctaaccgcttttttgcacaacatgggggatcatgtaactcgccttgatcgttgggaaccggagctgaatgaagccataccaaacgacgagcgtgacaccacgatgcctgtagcaatggcaacaacgttgcgcaaactattaactggcgaactacttactctagcttcccggcaacaattaatagactggatggaggcggataaagttgcaggaccacttctgcgctcggcccttccggctggctggtttattgctgataaatctggagccggtgagcgtgggtctcgcggtatcattgcagcactggggccagatggtaagccctcccgtatcgtagttatctacacgacggggagtcaggcaactatggatgaacgaaatagacagatcgctgagataggtgcctcactgattaagcattggtaactgtcagaccaagtttactcatatatactttagattgatttaaaacttcatttttaatttaaaaggatctaggtgaagatcctttttgataatctcatgaccaaaatcccttaacgtgagttttcgttccactgagcgtcagaccccgtagaaaagatcaaaggatcttcttgagatcctttttttctgcgcgtaatctgctgcttgcaaacaaaaaaaccaccgctaccagcggtggtttgtttgccggatcaagagctaccaactctttttccgaaggtaactggcttcagcagagcgcagataccaaatactgtccttctagtgtagccgtagttaggccaccacttcaagaactctgtagcaccgcctacatacctcgctctgctaatcctgttaccagtggctgctgccagtggcgataagtcgtgtcttaccgggttggactcaagacgatagttaccggataaggcgcagcggtcgggctgaacggggggttcgtgcacacagcccagcttggagcgaacgacctacaccgaactgagatacctacagcgtgagctatgagaaagcgccacgcttcccgaagggagaaaggcggacaggtatccggtaagcggcagggtcggaacaggagagcgcacgagggagcttccagggggaaacgcctggtatctttatagtcctgtcgggtttcgccacctctgacttgagcgtcgatttttgtgatgctcgtcaggggggcggagcctatggaaaaacgccagcaacgcggcctttttacggttcctggccttttgctggccttttgctcacatgttctttcctgcgttatcccctgattctgtggataaccgtattaccgcctttgagtgagctgataccgctcgccgcagccgaacgaccgagcgcagcgagtcagtgagcgaggaagcggaagagcgcccaatacgcaaaccgcctctccccgcgcgttggccgattcattaatgcagctgcgcgctcgctcgctcactgaggccgcccgggcaaagcccgggcgtcgggcgacctttggtcgcccggcctcagtgagcgagcgagcgcgcagagagggagtggccaactccatcactaggggttccttgtagttaatgattaacccgccatgctacttatctacgtagccatgctctagac

SEQ ID NO: 20 - DNA, 5930 bp, synthetic construct
  misc_feature 1..5930: note = pAAV mGAD67 (Rii-ETSS) GFP WPRE SV40pA
  misc_feature 2181: note = n is a, c, g, or t
  misc_feature 3452: note = n is a, c, g, or t
  source 1..5930: mol_type = other DNA
tcgagacaaaattcttcgtaggaattatattttcccttgccctcacccaacatcgcctatctcaaaaataatttaaaaacaaaaaacaaacaaacaaacaaaaaacagagcgtgctgagtgcattctggattactcataggactttgtcacacacaccctcctttctggtcgcaaacccgtgagctggatttataatcgccctacaaagctccagaggcagtcagacacctgcaaaggagccccagcgctccgcggacgagctgcccccgcgagcaacggcctcgtgattccccccgccgagcgggtccccgcctccccactccgcccccgcctcccccaagcccagcggccgcctctccggatctctcccttcttcaggctctcccgtgccggaccagggatcgtgcaagcaagaccggtcgccaccatggtgagcaagggcgaggagctgttcaccggggtggtgcccatcctggtcgagctggacggcgacgtaaacggccacaagttcagcgtgtccggcgagggcgagggcgatgccacctacggcaagctgaccctgaagttcatctgcaccaccggcaagctgcccgtgccctggcccaccctcgtgaccaccctgacctacggcgtgcagtgcttcagccgctaccccgaccacatgaagcagcacgacttcttcaagtccgccatgcccgaaggctacgtccaggagcgcaccatcttcttcaaggacgacggcaactacaagacccgcgccgaggtgaagttcgagggcgacaccctggtgaaccgcatcgagctgaagggcatcgacttcaaggaggacggcaacatcctggggcacaagctggagtacaactacaacagccacaacgtctatatcatggccgacaagcagaagaacggcatcaaggtgaacttcaagatccgccacaacatcgaggacggcagcgtgcagctcgccgaccactaccagcagaacacccccatcggcgacggccccgtgctgctgcccgacaaccactacctgagcacccagtccgccctgagcaaagaccccaacgagaagcgcgatcacatggtcctgctggagttcgtgaccgccgccgggatcactctcggcatggacgagctgtacaagtaaagcggccgcatcgataatcaacctctggattacaaaatttgtgaaagattgactggtattcttaactatgttgctccttttacgctatgtggatacgctgctttaatgcctttgtatcatgctattgcttcccgtatggctttcattttctcctccttgtataaatcctggttgctgtctctttatgaggagttgtggcccgttgtcaggcaacgtggcgtggtgtgcactgtgtttgctgacgcaacccccactggttggggcattgccaccacctgtcagctcctttccgggactttcgctttccccctccctattgccacggcggaactcatcgccgcctgccttgcccgctgctggacaggggctcggctgttgggcactgacaattccgtggtgttgtcggggaagctgacgtcctttccatggctgctcgcctgtgttgccacctggattctgcgcgggacgtccttctgctacgtcccttcggccctcaatccagcggaccttccttcccgcggcctgctgccggctctgcggcctcttccgcgtcttcgccttcgccctcagacgagtcggatctccctttgggccgcctccccgcatcgatgccgtatacggtaccacttgtttattgcagcttataatggttacaaataaagcaatagcatcacaaatttcacaaataaagcatttttttcactgcattctagttgtggtttgtccaaactcatcaatgtatcttatcatgtctgtcgacccccaacgcgttggagctctagagcatggctacgtagataagtagcatggcgggttaatcattaactacaaggaacccctagtgatggagttggccactccctctctgcgcgctcgctcgctcactgaggccgggcgaccaaaggtcgcccgacgcccgggctttgcccgggcggcctcagtgagcgagcgagcgcgcagctggcgtaatagcgaagaggcccgcaccgatcgcccttcccaacagttgcgcagcctgaatggcgaatggaanttccaacatccaataaatcatacaggcaaggcaaagaattagcaaaattaagcaataaagcctcagagcataaagctaaatcggttgtaccaaaaacattatgaccctgtaatacttttgcgggagaagcctttatttcaacgcaaggataaaaatttttagaaccctcatatattttaaatgcaatgcctgagtaatgtgtaggtaaagattcaaacgggtgagaaaggccggagacagtcaaatcaccatcaatatgatattcaaccgttctagctgataaattcatgccggagagggtagctatttttgagaggtctctacaaaggctatcaggtcattgcctgagagtctggagcaaacaagagaatcgatgaacggtaatcgtaaaactagcatgtcaatcatatgtaccccggttgataatcagaaaagccccaaaaacaggaagattgtataagcaaatatttaaattgtaaacgttaatattttgttaaaattcgcgttaaatttttgttaaatcagctcattttttaaccaataggccgaaatcggcaaaatcccttataaatcaaaagaatagaccgagatagggttgagtgttgttccagtttggaacaagagtccactattaaagaacgtggactccaacgtcaaagggcgaaaaaccgtctatcagggcgatggcccactacgtgaaccatcaccctaatcaagttttttggggtcgaggtgccgtaaagcactaaatcggaaccctaaagggagcccccgatttagagcttgacggggaaagccggcgaacgtggcgagaaaggaagggaagaaagcgaaaggagcgggcgctagggcgctggcaagtgtagcggtcacgctgcgcgtaaccaccacacccgccgcgcttaatgcgccgctacagggcgcgtactatggttgctttgacgagcacgtataacgtgctttcctcgttagaatcagagcgggagctaaacaggaggccgattaaagggattttagacaggaacggtacgccagaatcctgagaagtgtttttataatcagtgaggccaccgagtaaaagagtctgtccatcacgcaaattaaccgttgtcgcaatacttctttgattagtaataacatcacttgcctgagtagaagaactcaaactatcggccttgctggtaatatccagaacaatattaccgccagccattgcaacaggaaaaacgctcatggaaatacctacattttgacgctcaatcgtctggaanttcctgatgcggtattttctccttacgcatctgtgcggtatttcacaccgcatatggtgcactctcagtacaatctgctctgatgccgcatagttaagccagccccgacacccgccaacacccgctgacgcgccctgacgggcttgtctgctcccggcatccgcttacagacaagctgtgaccgtctccgggagctgcatgtgtcagaggttttcaccgtcatcaccgaaacgcgcgagacgaaagggcctcgtgatacgcctatttttataggttaatgtcatgataataatggtttcttagacgtcaggtggcacttttcggggaaatgtgcgcggaacccctatttgtttatttttctaaatacattcaaatatgtatccgctcatgagacaataaccctgataaatgcttcaataatattgaaaaaggaagagtatgagtattcaacatttccgtgtcgcccttattcccttttttgcggcattttgccttcctgtttttgctcacccagaaacgctggtgaaagtaaaagatgctgaagatcagttgggtgcacgagtgggttacatcgaactggatctcaacagcggtaagatccttgagagttttcgccccgaagaacgttttccaatgatgagcacttttaaagttctgctatgtggcgcggtattatcccgtattgacgccgggcaagagcaactcggtcgccgcatacactattctcagaatgacttggttgagtactcaccagtcacagaaaagcatcttacggatggcatgacagtaagagaattatgcagtgctgccataaccatgagtgataacactgcggccaacttacttctgacaacgatcggaggaccgaaggagctaaccgcttttttgcacaacatgggggatcatgtaactcgccttgatcgttgggaaccggagctgaatgaagccataccaaacgacgagcgtgacaccacgatgcctgtagcaatggcaacaacgttgcgcaaactattaactggcgaactacttactctagcttcccggcaacaattaatagactggatggaggcggataaagttgcaggaccacttctgcgctcggcccttccggctggctggtttattgctgataaatctggagccggtgagcgtgggtctcgcggtatcattgcagcactggggccagatggtaagccctcccgtatcgtagttatctacacgacggggagtcaggcaactatggatgaacgaaatagacagatcgctgagataggtgcctcactgattaagcattggtaactgtcagaccaagtttactcatatatactttagattgatttaaaacttcatttttaatttaaaaggatctaggtgaagatcctttttgataatctcatgaccaaaatcccttaacgtgagttttcgttccactgagcgtcagaccccgtagaaaagatcaaaggatcttcttgagatcctttttttctgcgcgtaatctgctgcttgcaaacaaaaaaaccaccgctaccagcggtggtttgtttgccggatcaagagctaccaactctttttccgaaggtaactggcttcagcagagcgcagataccaaatactgtccttctagtgtagccgtagttaggccaccacttcaagaactctgtagcaccgcctacatacctcgctctgctaatcctgttaccagtggctgctgccagtggcgataagtcgtgtcttaccgggttggactcaagacgatagttaccggataaggcgcagcggtcgggctgaacggggggttcgtgcacacagcccagcttggagcgaacgacctacaccgaactgagatacctacagcgtgagctatgagaaagcgccacgcttcccgaagggagaaaggcggacaggtatccggtaagcggcagggtcggaacaggagagcgcacgagggagcttccagggggaaacgcctggtatctttatagtcctgtcgggtttcgccacctctgacttgagcgtcgatttttgtgatgctcgtcaggggggcggagcctatggaaaaacgccagcaacgcggcctttttacggttcctggccttttgctggccttttgctcacatgttctttcctgcgttatcccctgattctgtggataaccgtattaccgcctttgagtgagctgataccgctcgccgcagccgaacgaccgagcgcagcgagtcagtgagcgaggaagcggaagagcgcccaatacgcaaaccgcctctccccgcgcgttggccgattcattaatgcagctgcgcgctcgctcgctcactgaggccgcccgggcaaagcccgggcgtcgggcgacctttggtcgcccggcctcagtgagcgagcgagcgcgcagagagggagtggccaactccatcactaggggttccttgtagttaatgattaacccgccatgctacttatctacgtagccatgctctagac

SEQ ID NO: 21 - DNA, 1061 bp, synthetic construct
  misc_feature 1..1061: note = template sequence of mGAD65(Ri-Rii-D)
  source 1..1061: mol_type = other DNA
atgctctagactcgagatttctgggtggctcacagtggacaaggaataggtaatcccaccaaaccttgaggtgggctaaactggagattttggtatgggtctcctactgtaaagagaaagccttccgggctaacggtattcctttcgcagtctactgcctcctttgtgaactaatgactgtaattattacctcccagagctcttttgttatcaacaacccggaggaaaagggaaacagaaaggattttttcattcctttattagaaaacacaaacgaaactacttctttctgggctgggaaattgccactgttgtgttcctaggcacctgctgatggcaagaactcctcttgggaagggacgaggtcagtgggttgagtatccctgaaaagatgggagtgccttttcctgggatttggaaaaactgattcgcttactttgagactccctgaatcctgtgtatgtgtcagctctcacccactccaagaagtttctgttcgttttatttatttaatttttctcagcctgaggtcctcagtgatagattccagcgtggattttaattgcttcaatcagcagcctttctcttcagccgtcagtcaaaacctggacgatgggtctggggacccaggcatgactgcacagaaaccgtacgacccccacccccaccccccaggctggctcagctcagcaggcagacattaggctctgctaaggagatgaaatgagttcgttggtgtggaagcggtccaccttcctccctccttggttccttccccaagctttggagctcttcctgattgaggccaggtggcctgggctcttgaggtcacagcgacctcagcactggtttggaggaaggcgggcgcgagaaccacttttgctcggcagcagccagagacagccctcaaacaatgagccaatcgatgcacacgtgaaattgccctcggccaccattccaatcttgccaaggtctccctgtccctggggtcacctaggccagcgtgctgagggctgtggtagcaccctggacagcgcgttccggcagaagcagacctggag

SEQ ID NO: 22 - DNA, 37 bp, synthetic construct
  misc_feature 1..37: note = forward primer for mGAD65(Ri-Rii-D)
  source 1..37: mol_type = other DNA
atgctctagactcgagatttctgggtggctcacagtg

SEQ ID NO: 23 - DNA, 36 bp, synthetic construct
  misc_feature 1..36: note = reverse primer for mGAD65(Ri-Rii-D)
  source 1..36: mol_type = other DNA
acccagccacaggcgctccaggtctgcttctgccgg

SEQ ID NO: 24 - DNA, 122 bp, synthetic construct; identical to SEQ ID NO: 3
  misc_feature 1..122: note = template sequence of mGAD65(ETSS)
  source 1..122: mol_type = other DNA

SEQ ID NO: 25 - DNA, 19 bp, synthetic construct
  misc_feature 1..19: note = forward primer for mGAD65(ETSS)
  source 1..19: mol_type = other DNA
cgcctgtggctgggtcagc

SEQ ID NO: 26 - DNA, 35 bp, synthetic construct
  misc_feature 1..35: note = reverse primer for mGAD65(ETSS)
  source 1..35: mol_type = other DNA
catggtggcgaccggtgagggagcttggtggggag

SEQ ID NO: 27 - DNA, 589 bp, synthetic construct
  misc_feature 1..589: note = template sequence of mGAD65(Ri-Rii)
  source 1..589: mol_type = other DNA
atgctctagactcgagatttctgggtggctcacagtggacaaggaataggtaatcccaccaaaccttgaggtgggctaaactggagattttggtatgggtctcctactgtaaagagaaagccttccgggctaacggtattcctttcgcagtctactgcctcctttgtgaactaatgactgtaattattacctcccagagctcttttgttatcaacaacccggaggaaaagggaaacagaaaggattttttcattcctttattagaaaacacaaacgaaactacttctttctgggctgggaaattgccactgttgtgttcctaggcacctgctgatggcaagaactcctcttgggaagggacgaggtcagtgggttgagtatccctgaaaagatgggagtgccttttcctgggatttggaaaaactgattcgcttactttgagactccctgaatcctgtgtatgtgtcagctctcacccactccaagaagtttctgttcgttttatttatttaatttttctcagcctgaggtcctcagtgatagattccagcgtggattttaattgcttcaatcagcagcctttctcttc

SEQ ID NO: 28 - DNA, 37 bp, synthetic construct; identical to SEQ ID NO: 22
  misc_feature 1..37: note = forward primer for mGAD65(Ri-Rii)
  source 1..37: mol_type = other DNA

SEQ ID NO: 29 - DNA, 35 bp, synthetic construct
  misc_feature 1..35: note = reverse primer for mGAD65(Ri-Rii)
  source 1..35: mol_type = other DNA
acccagccacaggcgaagagaaaggctgctgattg

SEQ ID NO: 30 - DNA, 505 bp, synthetic construct
  misc_feature 1..505: note = template sequence of mGAD65(Rii-ETSS)
  source 1..505: mol_type = other DNA
gaggaaaagggaaacagaaaggattttttcattcctttattagaaaacacaaacgaaactacttctttctgggctgggaaattgccactgttgtgttcctaggcacctgctgatggcaagaactcctcttgggaagggacgaggtcagtgggttgagtatccctgaaaagatgggagtgccttttcctgggatttggaaaaactgattcgcttactttgagactccctgaatcctgtgtatgtgtcagctctcacccactccaagaagtttctgttcgttttatttatttaatttttctcagcctgaggtcctcagtgatagattccagcgtggattttaattgcttcaatcagcagcctttctcttcgcctgtggctgggtcagcactacgcaggcacgcctccctcccccgcatctgactcgcacctcacgacccagcgcctccatttcccttccgtcactctctcatctccccaccaagctccctcaccggtcgccaccatg

SEQ ID NO: 31 - DNA, 43 bp, synthetic construct
  misc_feature 1..43: note = forward primer for mGAD65(Rii-ETSS)
  source 1..43: mol_type = other DNA
atgctctagactcgaggaaaagggaaacagaaaggattttttc

SEQ ID NO: 32 - DNA, 35 bp, synthetic construct; identical to SEQ ID NO: 26
  misc_feature 1..35: note = reverse primer for mGAD65(Rii-ETSS)
  source 1..35: mol_type = other DNA

SEQ ID NO: 33 - DNA, 967 bp, synthetic construct
  misc_feature 1..967: note = template sequence of mGAD67(Ri-M-Rii-ETSS)
  source 1..967: mol_type = other DNA
cttcaccccgctcagtaatgtgcttaaatattgccaagagagaatcattgaacagcgtgaaactgaaaagaagcgaggagagcgggccaagacacggagtgccgtcctggcttcccggagccaccctccatgctctgctgccccaggcgtgtggagcggcactcgtgcgtgttattaaccttcagacatgatcaattacgaagatttcttttacccctctccagggagagggctcagagaaagggaaatagaccccttgcctcttgtggtgccaggtagctgtgttcgaacgaggtagtgtggagatggactggaagaagaaacgggagtgcagaaactccagggtctgtctgggtggtcccctcatctccgctttgcctgtacagccatactggctcagtagagcgctccctaggacaccacccagagaaaaccttctggaatcgccaatccaggacaaccacaggagattgatcaaggcaaagcaaatattctagtcttctccaagatacgggatggagggctaggaagaggggaaggaagaatcacccagtgagacaaaattcttcgtaggaattatattttcccttgccctcacccaacatcgcctatctcaaaaataatttaaaaacaaaaaacaaacaaacaaacaaaaaacagagcgtgctgagtgcattctggattactcataggactttgtcacacacaccctcctttctggtcgcaaacccgtgagctggatttataatcgccctacaaagctccagaggcagtcagacacctgcaaaggagccccagcgctccgcggacgagctgcccccgcgagcaacggcctcgtgattccccccgccgagcgggtccccgcctccccactccgcccccgcctcccccaagcccagcggccgcctctccggatctctcccttcttcaggctctcccgtgccggaccagggatcgtgcaagcaag

SEQ ID NO: 34 - DNA, 36 bp, synthetic construct
  misc_feature 1..36: note = forward primer for mGAD67(Ri-M-Rii-ETSS)
  source 1..36: mol_type = other DNA
atgctctagactcgagcttcaccccgctcagtaatg

SEQ ID NO: 35 - DNA, 35 bp, synthetic construct
  misc_feature 1..35: note = reverse primer for mGAD67(Ri-M-Rii-ETSS)
  source 1..35: mol_type = other DNA
catggtggcgaccggtcttgcttgcacgatccctg

SEQ ID NO: 36 - DNA, 293 bp, synthetic construct
  misc_feature 1..293: note = template sequence of mGAD67(Ri)
  source 1..293: mol_type = other DNA
atgctctagactcgagcttcaccccgctcagtaatgtgcttaaatattgccaagagagaatcattgaacagcgtgaaactgaaaagaagcgaggagagcgggccaagacacggagtgccgtcctggcttcccggagccaccctccatgctctgctgccccaggcgtgtggagcggcactcgtgcgtgttattaaccttcagacatgatcaattacgaagatttcttttacccctctccagggagagggctcagagaaagggaaatagaccccttgcctcttgtggtgccaggt

SEQ ID NO: 37 - DNA, 36 bp, synthetic construct; identical to SEQ ID NO: 34
  misc_feature 1..36: note = forward primer for mGAD67(Ri)
  source 1..36: mol_type = other DNA

SEQ ID NO: 38 - DNA, 34 bp, synthetic construct
  misc_feature 1..34: note = reverse primer for mGAD67(Ri)
  source 1..34: mol_type = other DNA
acgaagaattttgtcacctggcaccacaagaggc

SEQ ID NO: 39 - DNA, 411 bp, synthetic construct
  misc_feature 1..411: note = template sequence of mGAD67(Rii-ETSS)
  source 1..411: mol_type = other DNA
gacaaaattcttcgtaggaattatattttcccttgccctcacccaacatcgcctatctcaaaaataatttaaaaacaaaaaacaaacaaacaaacaaaaaacagagcgtgctgagtgcattctggattactcataggactttgtcacacacaccctcctttctggtcgcaaacccgtgagctggatttataatcgccctacaaagctccagaggcagtcagacacctgcaaaggagccccagcgctccgcggacgagctgcccccgcgagcaacggcctcgtgattccccccgccgagcgggtccccgcctccccactccgcccccgcctcccccaagcccagcggccgcctctccggatctctcccttcttcaggctctcccgtgccggaccagggatcgtgcaagcaag

SEQ ID NO: 40 - DNA, 31 bp, synthetic construct
  misc_feature 1..31: note = forward primer for mGAD67(Rii-ETSS)
  source 1..31: mol_type = other DNA
gacaaaattcttcgtaggaattatattttcc

SEQ ID NO: 41 - DNA, 35 bp, synthetic construct; identical to SEQ ID NO: 35
  misc_feature 1..35: note = reverse primer for mGAD67(Rii-ETSS)
  source 1..35: mol_type = other DNA

SEQ ID NO: 42 - DNA, 427 bp, synthetic construct
  misc_feature 1..427: note = template sequence of mGAD67(Rii-ETSS)
  source 1..427: mol_type = other DNA
gacaaaattcttcgtaggaattatattttcccttgccctcacccaacatcgcctatctcaaaaataatttaaaaacaaaaaacaaacaaacaaacaaaaaacagagcgtgctgagtgcattctggattactcataggactttgtcacacacaccctcctttctggtcgcaaacccgtgagctggatttataatcgccctacaaagctccagaggcagtcagacacctgcaaaggagccccagcgctccgcggacgagctgcccccgcgagcaacggcctcgtgattccccccgccgagcgggtccccgcctccccactccgcccccgcctcccccaagcccagcggccgcctctccggatctctcccttcttcaggctctcccgtgccggaccagggatcgtgcaagcaagaccggtcgccaccatg

SEQ ID NO: 43 - DNA, 33 bp, synthetic construct
  misc_feature 1..33: note = forward primer for mGAD67(Rii-ETSS)
  source 1..33: mol_type = other DNA
atgctctagactcgagacaaaattcttcgtagg

SEQ ID NO: 44 - DNA, 35 bp, synthetic construct; identical to SEQ ID NO: 35
  misc_feature 1..35: note = reverse primer for mGAD67(Rii-ETSS)
  source 1..35: mol_type = other DNA

SEQ ID NO: 45 - DNA, 20 bp, synthetic construct
  misc_feature 1..20: note = WPRE forward primer
  source 1..20: mol_type = other DNA
ctgttgggcactgacaattc

SEQ ID NO: 46 - DNA, 20 bp, synthetic construct
  misc_feature 1..20: note = WPRE reverse primer
  source 1..20: mol_type = other DNA
gaagggacgtagcagaagga

SEQ ID NO: 47 - DNA, 20 bp, synthetic construct
  misc_feature 1..20: note = qRTPCR-mGAPDH-F
  source 1..20: mol_type = other DNA
gtgttcctacccccaatgtg

SEQ ID NO: 48 - DNA, 22 bp, synthetic construct
  misc_feature 1..22: note = qRTPCR-mGAPDH-R
  source 1..22: mol_type = other DNA
ggtggaagagtgggagttgctg

SEQ ID NO: 49 - DNA, 21 bp, synthetic construct
  misc_feature 1..21: note = qPCR-AAV-EGFP-F
  source 1..21: mol_type = other DNA
ggacgagctgtacaagtaaag

SEQ ID NO: 50 - DNA, 25 bp, synthetic construct
  misc_feature 1..25: note = qPCR-AAV-WPRE-R
  source 1..25: mol_type = other DNA
gggaagcaatagcatgatacaaagg